European Patent Specification EP 4 143 229 B1, published July 30, 2025. Title: ILT-BINDING AGENTS AND METHODS OF USE THEREOF. Applicant: NGM BIOPHARMACEUTICALS, INC. The sequence listing filed with the application follows.

SEQUENCE LISTING (173 sequences)

SEQ ID NO: 1 - protein, 650 aa, Homo sapiens
MTPILTVLICLGLSLGPRTHVQAGHLPKPTLWAEPGSVITQGSPVTLRCQGGQETQEYRLYREKKTALWITRIPQELVKKGQFPIPSITWEHAGRYRCYYGSDTAGRSESSDPLELVVTGAYIKPTLSAQPSPVVNSGGNVILQCDSQVAFDGFSLCKEGEDEHPQCLNSQPHARGSSRAIFSVGPVSPSRRWWYRCYAYDSNSPYEWSLPSDLLELLVLGVSKKPSLSVQPGPIVAPEETLTLQCGSDAGYNRFVLYKDGERDFLQLAGAQPQAGLSQANFTLGPVSRSYGGQYRCYGAHNLSSEWSAPSDPLDILIAGQFYDRVSLSVQPGPTVASGENVTLLCQSQGWMQTFLLTKEGAADDPWRLRSTYQSQKYQAEFPMGPVTSAHAGTYRCYGSQSSKPYLLTHPSDPLELVVSGPSGGPSSPTTGPTSTSGPEDQPLTPTGSDPQSGLGRHLGVVIGILVAVILLLLLLLLLFLILRHRRQGKHWTSTQRKADFQHPAGAVGPEPTDRGLQWRSSPAADAQEENLYAAVKHTQPEDGVEMDTRSPHDEDPQAVTYAEVKHSRPRREMASPPSPLSGEFLDTKDRQAEEDRQMDTEAAASEAPQDVTYAQLHSLTLRREATEPPPSQEGPSPAVPSIYATLAIH

SEQ ID NO: 2 - protein, 627 aa, Homo sapiens
GHLPKPTLWAEPGSVITQGSPVTLRCQGGQETQEYRLYREKKTALWITRIPQELVKKGQFPIPSITWEHAGRYRCYYGSDTAGRSESSDPLELVVTGAYIKPTLSAQPSPVVNSGGNVILQCDSQVAFDGFSLCKEGEDEHPQCLNSQPHARGSSRAIFSVGPVSPSRRWWYRCYAYDSNSPYEWSLPSDLLELLVLGVSKKPSLSVQPGPIVAPEETLTLQCGSDAGYNRFVLYKDGERDFLQLAGAQPQAGLSQANFTLGPVSRSYGGQYRCYGAHNLSSEWSAPSDPLDILIAGQFYDRVSLSVQPGPTVASGENVTLLCQSQGWMQTFLLTKEGAADDPWRLRSTYQSQKYQAEFPMGPVTSAHAGTYRCYGSQSSKPYLLTHPSDPLELVVSGPSGGPSSPTTGPTSTSGPEDQPLTPTGSDPQSGLGRHLGVVIGILVAVILLLLLLLLLFLILRHRRQGKHWTSTQRKADFQHPAGAVGPEPTDRGLQWRSSPAADAQEENLYAAVKHTQPEDGVEMDTRSPHDEDPQAVTYAEVKHSRPRREMASPPSPLSGEFLDTKDRQAEEDRQMDTEAAASEAPQDVTYAQLHSLTLRREATEPPPSQEGPSPAVPSIYATLAIH

SEQ ID NO: 3 - protein, 438 aa, Homo sapiens
GHLPKPTLWAEPGSVITQGSPVTLRCQGGQETQEYRLYREKKTALWITRIPQELVKKGQFPIPSITWEHAGRYRCYYGSDTAGRSESSDPLELVVTGAYIKPTLSAQPSPVVNSGGNVILQCDSQVAFDGFSLCKEGEDEHPQCLNSQPHARGSSRAIFSVGPVSPSRRWWYRCYAYDSNSPYEWSLPSDLLELLVLGVSKKPSLSVQPGPIVAPEETLTLQCGSDAGYNRFVLYKDGERDFLQLAGAQPQAGLSQANFTLGPVSRSYGGQYRCYGAHNLSSEWSAPSDPLDILIAGQFYDRVSLSVQPGPTVASGENVTLLCQSQGWMQTFLLTKEGAADDPWRLRSTYQSQKYQAEFPMGPVTSAHAGTYRCYGSQSSKPYLLTHPSDPLELVVSGPSGGPSSPTTGPTSTSGPEDQPLTPTGSDPQSGLGRHLGV

SEQ ID NO: 4 - protein, 89 aa, Homo sapiens
PKPTLWAEPGSVITQGSPVTLRCQGGQETQEYRLYREKKTALWITRIPQELVKKGQFPIPSITWEHAGRYRCYYGSDTAGRSESSDPLE

SEQ ID NO: 5 - protein, 106 aa, Homo sapiens
LVVTGAYIKPTLSAQPSPVVNSGGNVILQCDSQVAFDGFSLCKEGEDEHPQCLNSQPHARGSSRAIFSVGPVSPSRRWWYRCYAYDSNSPYEWSLPSDLLELLVLG

SEQ ID NO: 6 - protein, 91 aa, Homo sapiens
VSKKPSLSVQPGPIVAPEETLTLQCGSDAGYNRFVLYKDGERDFLQLAGAQPQAGLSQANFTLGPVSRSYGGQYRCYGAHNLSSEWSAPSD

SEQ ID NO: 7 - protein, 97 aa, Homo sapiens
PLDILIAGQFYDRVSLSVQPGPTVASGENVTLLCQSQGWMQTFLLTKEGAADDPWRLRSTYQSQKYQAEFPMGPVTSAHAGTYRCYGSQSSKPYLLT

SEQ ID NO: 8 - protein, 598 aa, Homo sapiens
MTPIVTVLICLGLSLGPRTHVQTGTIPKPTLWAEPDSVITQGSPVTLSCQGSLEAQEYRLYREKKSASWITRIRPELVKNGQFHIPSITWEHTGRYGCQYYSRARWSELSDPLVLVMTGAYPKPTLSAQPSPVVTSGGRVTLQCESQVAFGGFILCKEGEEEHPQCLNSQPHARGSSRAIFSVGPVSPNRRWSHRCYGYDLNSPYVWSSPSDLLELLVPGVSKKPSLSVQPGPVVAPGESLTLQCVSDVGYDRFVLYKEGERDLRQLPGRQPQAGLSQANFTLGPVSRSYGGQYRCYGAHNLSSECSAPSDPLDILITGQIRGTPFISVQPGPTVASGENVTLLCQSWRQFHTFLLTKAGAADAPLRLRSIHEYPKYQAEFPMSPVTSAHAGTYRCYGSLNSDPYLLSHPSEPLELVVSGPSMGSSPPPTGPISTPAGPEDQPLTPTGSDPQSGLGRHLGVVIGILVAVVLLLLLLLLLFLILRHRRQGKHWTSTQRKADFQHPAGAVGPEPTDRGLQWRSSPAADAQEENLYAAVKDTQPEDGVEMDTRAAASEAPQDVTYAQLHSLTLRRKATEPPPSQEREPPAEPSIYATLAIH

SEQ ID NO: 9 - protein, 577 aa, Homo sapiens
QTGTIPKPTLWAEPDSVITQGSPVTLSCQGSLEAQEYRLYREKKSASWITRIRPELVKNGQFHIPSITWEHTGRYGCQYYSRARWSELSDPLVLVMTGAYPKPTLSAQPSPVVTSGGRVTLQCESQVAFGGFILCKEGEEEHPQCLNSQPHARGSSRAIFSVGPVSPNRRWSHRCYGYDLNSPYVWSSPSDLLELLVPGVSKKPSLSVQPGPVVAPGESLTLQCVSDVGYDRFVLYKEGERDLRQLPGRQPQAGLSQANFTLGPVSRSYGGQYRCYGAHNLSSECSAPSDPLDILITGQIRGTPFISVQPGPTVASGENVTLLCQSWRQFHTFLLTKAGAADAPLRLRSIHEYPKYQAEFPMSPVTSAHAGTYRCYGSLNSDPYLLSHPSEPLELVVSGPSMGSSPPPTGPISTPAGPEDQPLTPTGSDPQSGLGRHLGVVIGILVAVVLLLLLLLLLFLILRHRRQGKHWTSTQRKADFQHPAGAVGPEPTDRGLQWRSSPAADAQEENLYAAVKDTQPEDGVEMDTRAAASEAPQDVTYAQLHSLTLRRKATEPPPSQEREPPAEPSIYATLAIH

SEQ ID NO: 10 - protein, 440 aa, Homo sapiens
QTGTIPKPTLWAEPDSVITQGSPVTLSCQGSLEAQEYRLYREKKSASWITRIRPELVKNGQFHIPSITWEHTGRYGCQYYSRARWSELSDPLVLVMTGAYPKPTLSAQPSPVVTSGGRVTLQCESQVAFGGFILCKEGEEEHPQCLNSQPHARGSSRAIFSVGPVSPNRRWSHRCYGYDLNSPYVWSSPSDLLELLVPGVSKKPSLSVQPGPVVAPGESLTLQCVSDVGYDRFVLYKEGERDLRQLPGRQPQAGLSQANFTLGPVSRSYGGQYRCYGAHNLSSECSAPSDPLDILITGQIRGTPFISVQPGPTVASGENVTLLCQSWRQFHTFLLTKAGAADAPLRLRSIHEYPKYQAEFPMSPVTSAHAGTYRCYGSLNSDPYLLSHPSEPLELVVSGPSMGSSPPPTGPISTPAGPEDQPLTPTGSDPQSGLGRHLGV

SEQ ID NO: 11 - protein, 84 aa, Homo sapiens
PKPTLWAEPDSVITQGSPVTLSCQGSLEAQEYRLYREKKSASWITRIRPELVKNGQFHIPSITWEHTGRYGCQYYSRARWSELS

SEQ ID NO: 12 - protein, 119 aa, Homo sapiens
DPLVLVMTGAYPKPTLSAQPSPVVTSGGRVTLQCESQVAFGGFILCKEGEEEHPQCLNSQPHARGSSRAIFSVGPVSPNRRWSHRCYGYDLNSPYVWSSPSDLLELLVPGVSKKPSLSV

SEQ ID NO: 13 - protein, 89 aa, Homo sapiens
QPGPVVAPGESLTLQCVSDVGYDRFVLYKEGERDLRQLPGRQPQAGLSQANFTLGPVSRSYGGQYRCYGAHNLSSECSAPSDPLDILIT

SEQ ID NO: 14 - protein, 90 aa, Homo sapiens
QPGPTVASGENVTLLCQSWRQFHTFLLTKAGAADAPLRLRSIHEYPKYQAEFPMSPVTSAHAGTYRCYGSLNSDPYLLSHPSEPLELVVS

SEQ ID NO: 15 - protein, 639 aa, Macaca mulatta
  MOD_RES (150)..(150): Any amino acid
MTPILMVLICLGLSLGSRTRVQAGTFPKPTLWAEPGSMISKGSPVTLRCQGSLPVQDYRLQREKKTASWVRRIQQELVKKGYFPIASITSEHAGQYRCQYYSHSWWSEPSDPLELVVTGAYSKPTLSALPSPVVASGGNVTLQCDSQVAXGGFVLCKEGEDEHPQCLNSQPHTRGSSRAVFSVGPVSPSRRWSYRCYGYDSRSPYVWSLPSDLLELLVPGVSKKPSLSVQPGPVVAPGDKLTLQCGSDAGYNRFALYKEGERDFLQRPGRQPQAGLSQANFLLDPVRRSHGGQYRCSGAHNLSSEWSAPSDPLDILIAGQIRGRPSLLVQPGPTVVSGENVTLLCQSSWQFHVFLLTQAGAADAHLHLRSMYKYPKYQAEFPMSPVTSAHAGTYRCYGSHSSDSYLLSIPSDPLELVVSGPSGGPSSPTTGPTSTCGPEDQPLTPTGSDPQSGLGRHLGVVTGVLVAFVLLLFLLLLLFLVLRHRRQGKRWTSAQRKADFQHPAGAVEPEPRDRGLQRRSSPAANTQEENLYAAVKDTQPEDGVELDSRSPHDEDPQAVTYARVKHSRPRREMASPPSPLSEEFLDTKDTQAAASEDPQDVTYAQLQSLTLRRETTEPPPSQEREPPVESSIYATLTIH

SEQ ID NO: 16 - protein, 616 aa, Macaca mulatta
  MOD_RES (127)..(127): Any amino acid
GTFPKPTLWAEPGSMISKGSPVTLRCQGSLPVQDYRLQREKKTASWVRRIQQELVKKGYFPIASITSEHAGQYRCQYYSHSWWSEPSDPLELVVTGAYSKPTLSALPSPVVASGGNVTLQCDSQVAXGGFVLCKEGEDEHPQCLNSQPHTRGSSRAVFSVGPVSPSRRWSYRCYGYDSRSPYVWSLPSDLLELLVPGVSKKPSLSVQPGPVVAPGDKLTLQCGSDAGYNRFALYKEGERDFLQRPGRQPQAGLSQANFLLDPVRRSHGGQYRCSGAHNLSSEWSAPSDPLDILIAGQIRGRPSLLVQPGPTVVSGENVTLLCQSSWQFHVFLLTQAGAADAHLHLRSMYKYPKYQAEFPMSPVTSAHAGTYRCYGSHSSDSYLLSIPSDPLELVVSGPSGGPSSPTTGPTSTCGPEDQPLTPTGSDPQSGLGRHLGVVTGVLVAFVLLLFLLLLLFLVLRHRRQGKRWTSAQRKADFQHPAGAVEPEPRDRGLQRRSSPAANTQEENLYAAVKDTQPEDGVELDSRSPHDEDPQAVTYARVKHSRPRREMASPPSPLSEEFLDTKDTQAAASEDPQDVTYAQLQSLTLRRETTEPPPSQEREPPVESSIYATLTIH

SEQ ID NO: 17 - protein, 437 aa, Macaca mulatta
  MOD_RES (127)..(127): Any amino acid
GTFPKPTLWAEPGSMISKGSPVTLRCQGSLPVQDYRLQREKKTASWVRRIQQELVKKGYFPIASITSEHAGQYRCQYYSHSWWSEPSDPLELVVTGAYSKPTLSALPSPVVASGGNVTLQCDSQVAXGGFVLCKEGEDEHPQCLNSQPHTRGSSRAVFSVGPVSPSRRWSYRCYGYDSRSPYVWSLPSDLLELLVPGVSKKPSLSVQPGPVVAPGDKLTLQCGSDAGYNRFALYKEGERDFLQRPGRQPQAGLSQANFLLDPVRRSHGGQYRCSGAHNLSSEWSAPSDPLDILIAGQIRGRPSLLVQPGPTVVSGENVTLLCQSSWQFHVFLLTQAGAADAHLHLRSMYKYPKYQAEFPMSPVTSAHAGTYRCYGSHSSDSYLLSIPSDPLELVVSGPSGGPSSPTTGPTSTCGPEDQPLTPTGSDPQSGLGRHLGV

SEQ ID NO: 18 - protein, 88 aa, Macaca mulatta
PKPTLWAEPGSMISKGSPVTLRCQGSLPVQDYRLQREKKTASWVRRIQQELVKKGYFPIASITSEHAGQYRCQYYSHSWWSEPSDPLE

SEQ ID NO: 19 - protein, 106 aa, Macaca mulatta
  MOD_RES (36)..(36): Any amino acid
LVVTGAYSKPTLSALPSPVVASGGNVTLQCDSQVAXGGFVLCKEGEDEHPQCLNSQPHTRGSSRAVFSVGPVSPSRRWSYRCYGYDSRSPYVWSLPSDLLELLVPG

SEQ ID NO: 20 - protein, 91 aa, Macaca mulatta
VSKKPSLSVQPGPVVAPGDKLTLQCGSDAGYNRFALYKEGERDFLQRPGRQPQAGLSQANFLLDPVRRSHGGQYRCSGAHNLSSEWSAPSD

SEQ ID NO: 21 - protein, 97 aa, Macaca mulatta
PLDILIAGQIRGRPSLLVQPGPTVVSGENVTLLCQSSWQFHVFLLTQAGAADAHLHLRSMYKYPKYQAEFPMSPVTSAHAGTYRCYGSHSSDSYLLS

SEQ ID NO: 22 - protein, 10 aa, Artificial Sequence
  source: /note="Description of Artificial Sequence: Synthetic peptide"
GFSLTNYGVS

SEQ ID NO: 23 - protein, 16 aa, Artificial Sequence
  source: /note="Description of Artificial Sequence: Synthetic peptide"
IIWGDGSTNYHSALIS

SEQ ID NO: 24 - protein, 10 aa, Artificial Sequence
  source: /note="Description of Artificial Sequence: Synthetic peptide"
PNWDTYAMDF

SEQ ID NO: 25 - protein, 11 aa, Artificial Sequence
  source: /note="Description of Artificial Sequence: Synthetic peptide"
RASQDISNFLN

SEQ ID NO: 26 - protein, 7 aa, Artificial Sequence
  source: /note="Description of Artificial Sequence: Synthetic peptide"
CTSKLHS

SEQ ID NO: 27 - protein, 9 aa, Artificial Sequence
  source: /note="Description of Artificial Sequence: Synthetic peptide"
QQGNTLPPT

SEQ ID NO: 28 - protein, 7 aa, Artificial Sequence
  source: /note="Description of Artificial Sequence: Synthetic peptide"
GFSLTNY

SEQ ID NO: 29 - protein, 5 aa, Artificial Sequence
  source: /note="Description of Artificial Sequence: Synthetic peptide"
WGDGS

SEQ ID NO: 30 - protein, 9 aa, Artificial Sequence
  source: /note="Description of Artificial Sequence: Synthetic peptide"
IIWGDGSTN

SEQ ID NO: 31 - protein, 5 aa, Artificial Sequence
  source: /note="Description of Artificial Sequence: Synthetic peptide"
NYGVS

SEQ ID NO: 32 - protein, 6 aa, Artificial Sequence
  source: /note="Description of Artificial Sequence: Synthetic peptide"
TNYGVS

SEQ ID NO: 33 - protein, 12 aa, Artificial Sequence
  source: /note="Description of Artificial Sequence: Synthetic peptide"
WLGIIWGDGSTN

SEQ ID NO: 34 - protein, 11 aa, Artificial Sequence
  source: /note="Description of Artificial Sequence: Synthetic peptide"
AKPNWDTYAMD

SEQ ID NO: 35 - protein, 7 aa, Artificial Sequence
  source: /note="Description of Artificial Sequence: Synthetic peptide"
SNFLNWY

SEQ ID NO: 36 - protein, 10 aa, Artificial Sequence
  source: /note="Description of Artificial Sequence: Synthetic peptide"
LLIYCTSKLH

SEQ ID NO: 37 - protein, 8 aa, Artificial Sequence
  source: /note="Description of Artificial Sequence: Synthetic peptide"
QQGNTLPP

SEQ ID NO: 38 - protein, 10 aa, Artificial Sequence
  source: /note="Description of Artificial Sequence: Synthetic peptide"
GYSFTGYYMH

SEQ ID NO: 39 - protein, 17 aa, Artificial Sequence
  source: /note="Description of Artificial Sequence: Synthetic peptide"
RVYPNNGDTSYNQKFKV

SEQ ID NO: 40 - protein, 11 aa, Artificial Sequence
  source: /note="Description of Artificial Sequence: Synthetic peptide"
GATVVESLFAY

SEQ ID NO: 41 - protein, 15 aa, Artificial Sequence
  source: /note="Description of Artificial Sequence: Synthetic peptide"
RASESVDNYGNNFLH

SEQ ID NO: 42 - protein, 7 aa, Artificial Sequence
  source: /note="Description of Artificial Sequence: Synthetic peptide"
RTSNLES

SEQ ID NO: 43 - protein, 9 aa, Artificial Sequence
  source: /note="Description of Artificial Sequence: Synthetic peptide"
QQSNEDPYT

SEQ ID NO: 44 - protein, 7 aa, Artificial Sequence
  source: /note="Description of Artificial Sequence: Synthetic peptide"
GYSFTGY

SEQ ID NO: 45 - protein, 6 aa, Artificial Sequence
  source: /note="Description of Artificial Sequence: Synthetic peptide"
YPNNGD

SEQ ID NO: 46 - protein, 10 aa, Artificial Sequence
  source: /note="Description of Artificial Sequence: Synthetic peptide"
RVYPNNGDTS

SEQ ID NO: 47 - protein, 5 aa, Artificial Sequence
  source: /note="Description of Artificial Sequence: Synthetic peptide"
GYYMH

SEQ ID NO: 48 - protein, 6 aa, Artificial Sequence
  source: /note="Description of Artificial Sequence: Synthetic peptide"
TGYYMH

SEQ ID NO: 49 - protein, 13 aa, Artificial Sequence
  source: /note="Description of Artificial Sequence: Synthetic peptide"
WIGRVYPNNGDTS

SEQ ID NO: 50 - protein, 12 aa, Artificial Sequence
  source: /note="Description of Artificial Sequence: Synthetic peptide"
ARGATVVESLFA

SEQ ID NO: 51 - protein, 11 aa, Artificial Sequence
  source: /note="Description of Artificial Sequence: Synthetic peptide"
DNYGNNFLHWY

SEQ ID NO: 52 - protein, 10 aa, Artificial Sequence
  source: /note="Description of Artificial Sequence: Synthetic peptide"
LLIYRTSNLE

SEQ ID NO: 53 - protein, 8 aa, Artificial Sequence
  source: /note="Description of Artificial Sequence: Synthetic peptide"
QQSNEDPY

SEQ ID NO: 54 - protein, 10 aa, Artificial Sequence
  source: /note="Description of Artificial Sequence: Synthetic peptide"
GYTFTNYGMN

SEQ ID NO: 55 - protein, 17 aa, Artificial Sequence
  source: /note="Description of Artificial Sequence: Synthetic peptide"
WINTYIGEPIYADDFKG

SEQ ID NO: 56 - protein, 11 aa, Artificial Sequence
  source: /note="Description of Artificial Sequence: Synthetic peptide"
RSDYDGYAMDY

SEQ ID NO: 57 - protein, 17 aa, Artificial Sequence
  source: /note="Description of Artificial Sequence: Synthetic peptide"
KSSQSLLYSGNQKNYLA

SEQ ID NO: 58 - protein, 7 aa, Artificial Sequence
  source: /note="Description of Artificial Sequence: Synthetic peptide"
WASTRES

SEQ ID NO: 59 - protein, 8 aa, Artificial Sequence
  source: /note="Description of Artificial Sequence: Synthetic peptide"
QQHDSYPT

SEQ ID NO: 60 - protein, 7 aa, Artificial Sequence
  source: /note="Description of Artificial Sequence: Synthetic peptide"
GYTFTNY

SEQ ID NO: 61 - protein, 6 aa, Artificial Sequence
  source: /note="Description of Artificial Sequence: Synthetic peptide"
NTYIGE

SEQ ID NO: 62 - protein, 10 aa, Artificial Sequence
  source: /note="Description of Artificial Sequence: Synthetic peptide"
WINTYIGEPI

SEQ ID NO: 63 - protein, 5 aa, Artificial Sequence
  source: /note="Description of Artificial Sequence: Synthetic peptide"
NYGMN

SEQ ID NO: 64 - protein, 6 aa, Artificial Sequence
  source: /note="Description of Artificial Sequence: Synthetic peptide"
TNYGMN

SEQ ID NO: 65 - protein, 13 aa, Artificial Sequence
  source: /note="Description of Artificial Sequence: Synthetic peptide"
WMGWINTYIGEPI

SEQ ID NO: 66 - protein, 12 aa, Artificial Sequence
  source: /note="Description of Artificial Sequence: Synthetic peptide"
ARRSDYDGYAMD

SEQ ID NO: 67 - protein, 13 aa, Artificial Sequence
  source: /note="Description of Artificial Sequence: Synthetic peptide"
LYSGNQKNYLAWY

SEQ ID NO: 68 - protein, 10 aa, Artificial Sequence
  source: /note="Description of Artificial Sequence: Synthetic peptide"
LLIYWASTRE

SEQ ID NO: 69 - protein, 7 aa, Artificial Sequence
  source: /note="Description of Artificial Sequence: Synthetic peptide"
QQHDSYP

SEQ ID NO: 70 - protein, 10 aa, Artificial Sequence
  source: /note="Description of Artificial Sequence: Synthetic peptide"
GYTFTDYYMN

SEQ ID NO: 71 - protein, 17 aa, Artificial Sequence
  source: /note="Description of Artificial Sequence: Synthetic peptide"
DFNPNNGGTTYNQKFEG

SEQ ID NO: 72 - protein, 13 aa, Artificial Sequence
  source: /note="Description of Artificial Sequence: Synthetic peptide"
GRFYYGSLYSFDY

SEQ ID NO: 73 - protein, 11 aa, Artificial Sequence
  source: /note="Description of Artificial Sequence: Synthetic peptide"
RASGNIHNYLA

SEQ ID NO: 74 - protein, 7 aa, Artificial Sequence
  source: /note="Description of Artificial Sequence: Synthetic peptide"
NAKTLAD

SEQ ID NO: 75 - protein, 8 aa, Artificial Sequence
  source: /note="Description of Artificial Sequence: Synthetic peptide"
QHFWTSIT

SEQ ID NO: 76 - protein, 7 aa, Artificial Sequence
  source: /note="Description of Artificial Sequence: Synthetic peptide"
GYTFTDY

SEQ ID NO: 77 - protein, 6 aa, Artificial Sequence
  source: /note="Description of Artificial Sequence: Synthetic peptide"
NPNNGG

SEQ ID NO: 78 - protein, 10 aa, Artificial Sequence
  source: /note="Description of Artificial Sequence: Synthetic peptide"
DFNPNNGGTT

SEQ ID NO: 79 - protein, 5 aa, Artificial Sequence
  source: /note="Description of Artificial Sequence: Synthetic peptide"
DYYMN

SEQ ID NO: 80 - protein, 6 aa, Artificial Sequence
  source: /note="Description of Artificial Sequence: Synthetic peptide"
TDYYMN

SEQ ID NO: 81 - protein, 13 aa, Artificial Sequence
  source: /note="Description of Artificial Sequence: Synthetic peptide"
WIGDFNPNNGGTT

SEQ ID NO: 82 - protein, 14 aa, Artificial Sequence
  source: /note="Description of Artificial Sequence: Synthetic peptide"
ARGRFYYGSLYSFD

SEQ ID NO: 83 - protein, 7 aa, Artificial Sequence
  source: /note="Description of Artificial Sequence: Synthetic peptide"
HNYLAWY

SEQ ID NO: 84 - protein, 10 aa, Artificial Sequence
  source: /note="Description of Artificial Sequence: Synthetic peptide"
LLVYNAKTLA

SEQ ID NO: 85 - protein, 7 aa, Artificial Sequence
  source: /note="Description of Artificial Sequence: Synthetic peptide"
QHFWTSI

SEQ ID NO: 86 - protein, 10 aa, Artificial Sequence
  source: /note="Description of Artificial Sequence: Synthetic peptide"
GFTFNTYAMH

SEQ ID NO: 87 - protein, 19 aa, Artificial Sequence
  source: /note="Description of Artificial Sequence: Synthetic peptide"
RIRSKSSNYATYYADSVKD

SEQ ID NO: 88 - protein, 16 aa, Artificial Sequence
  source: /note="Description of Artificial Sequence: Synthetic peptide"
DGIYYYGTMYYYAMDY

SEQ ID NO: 89 - protein, 15 aa, Artificial Sequence
  source: /note="Description of Artificial Sequence: Synthetic peptide"
RASESVDYYGNSFMY

SEQ ID NO: 90 - protein, 7 aa, Artificial Sequence
  source: /note="Description of Artificial Sequence: Synthetic peptide"
FASNLES

SEQ ID NO: 91 - protein, 9 aa, Artificial Sequence
  source: /note="Description of Artificial Sequence: Synthetic peptide"
QQNNEDPWT

SEQ ID NO: 92 - protein, 7 aa, Artificial Sequence
  source: /note="Description of Artificial Sequence: Synthetic peptide"
GFTFNTY

SEQ ID NO: 93 - protein, 8 aa, Artificial Sequence
  source: /note="Description of Artificial Sequence: Synthetic peptide"
RSKSSNYA

SEQ ID NO: 94 - protein, 12 aa, Artificial Sequence
  source: /note="Description of Artificial Sequence: Synthetic peptide"
RIRSKSSNYATY

SEQ ID NO: 95 - protein, 5 aa, Artificial Sequence
  source: /note="Description of Artificial Sequence: Synthetic peptide"
TYAMH

SEQ ID NO: 96 - protein, 6 aa, Artificial Sequence
  source: /note="Description of Artificial Sequence: Synthetic peptide"
NTYAMH

SEQ ID NO: 97 - protein, 15 aa, Artificial Sequence
  source: /note="Description of Artificial Sequence: Synthetic peptide"
WVARIRSKSSNYATY

SEQ ID NO: 98 - protein, 17 aa, Artificial Sequence
  source: /note="Description of Artificial Sequence: Synthetic peptide"
VRDGIYYYGTMYYYAMD

SEQ ID NO: 99 - protein, 11 aa, Artificial Sequence
  source: /note="Description of Artificial Sequence: Synthetic peptide"
DYYGNSFMYWY

SEQ ID NO: 100 - protein, 10 aa, Artificial Sequence
  source: /note="Description of Artificial Sequence: Synthetic peptide"
LLIYFASNLE

SEQ ID NO: 101 - protein, 8 aa, Artificial Sequence
  source: /note="Description of Artificial Sequence: Synthetic peptide"
QQNNEDPW

SEQ ID NO: 102 - protein, 16 aa, Artificial Sequence
  source: /note="Description of Artificial Sequence: Synthetic peptide"
DGIYYYDTMYYYAMDY

SEQ ID NO: 103 - protein, 15 aa, Artificial Sequence
  source: /note="Description of Artificial Sequence: Synthetic peptide"
RASESVDYYGNSFIY

SEQ ID NO: 104 - protein, 17 aa, Artificial Sequence
  source: /note="Description of Artificial Sequence: Synthetic peptide"
VRDGIYYYDTMYYYAMD

SEQ ID NO: 105 - protein, 11 aa, Artificial Sequence
  source: /note="Description of Artificial Sequence: Synthetic peptide"
DYYGNSFIYWY

SEQ ID NO: 106 - protein, 17 aa, Artificial Sequence
  source: /note="Description of Artificial Sequence: Synthetic peptide"
NVNPNNGGTSYNQKFKG

SEQ ID NO: 107 - protein, 16 aa, Artificial Sequence
  source: /note="Description of Artificial Sequence: Synthetic peptide"
REIYFYGTIYYYAMDY

SEQ ID NO: 108 - protein, 10 aa, Artificial Sequence
  source: /note="Description of Artificial Sequence: Synthetic peptide"
NVNPNNGGTS

SEQ ID NO: 109 - protein, 13 aa, Artificial Sequence
  source: /note="Description of Artificial Sequence: Synthetic peptide"
WIGNVNPNNGGTS

SEQ ID NO: 110 - protein, 17 aa, Artificial Sequence
  source: /note="Description of Artificial Sequence: Synthetic peptide"
ARREIYFYGTIYYYAMD

SEQ ID NO: 111 - protein, 10 aa, Artificial Sequence
  source: /note="Description of Artificial Sequence: Synthetic peptide"
GYTFTDYYIN

SEQ ID NO: 112 - protein, 17 aa, Artificial Sequence
  source: /note="Description of Artificial Sequence: Synthetic peptide"
NVNPNDGGTTYNQKFKG

SEQ ID NO: 113 - protein, 6 aa, Artificial Sequence
  source: /note="Description of Artificial Sequence: Synthetic peptide"
NPNDGG

SEQ ID NO: 114 - protein, 10 aa, Artificial Sequence
  source: /note="Description of Artificial Sequence: Synthetic peptide"
NVNPNDGGTT

SEQ ID NO: 115 - protein, 5 aa, Artificial Sequence
  source: /note="Description of Artificial Sequence: Synthetic peptide"
DYYIN

SEQ ID NO: 116 - protein, 6 aa, Artificial Sequence
  source: /note="Description of Artificial Sequence: Synthetic peptide"
TDYYIN

SEQ ID NO: 117 - protein, 13 aa, Artificial Sequence
  source: /note="Description of Artificial Sequence: Synthetic peptide"
WIGNVNPNDGGTT

SEQ ID NO: 118 - protein, 17 aa, Artificial Sequence
  source: /note="Description of Artificial Sequence: Synthetic peptide"
DFNPNNAGTTYNQKFEG

SEQ ID NO: 119 - protein, 6 aa, Artificial Sequence
  source: /note="Description of Artificial Sequence: Synthetic peptide"
NPNNAG

SEQ ID NO: 120 - protein, 10 aa, Artificial Sequence
  source: /note="Description of Artificial Sequence: Synthetic peptide"
DFNPNNAGTT

SEQ ID NO: 121 - protein, 13 aa, Artificial Sequence
  source: /note="Description of Artificial Sequence: Synthetic peptide"
WIGDFNPNNAGTT

SEQ ID NO: 122 - protein, 10 aa, Artificial Sequence
  source: /note="Description of Artificial Sequence: Synthetic peptide"
LLIYNAKTLA

SEQ ID NO: 123 - protein, 17 aa, Artificial Sequence
  source: /note="Description of Artificial Sequence: Synthetic peptide"
ARDGIYYYDTMYYYAMD

SEQ ID NO: 124 - protein, 13 aa, Artificial Sequence
  source: /note="Description of Artificial Sequence: Synthetic peptide"
WMGNVNPNDGGTT

SEQ ID NO: 125 - protein, 118 aa, Artificial Sequence
  source: /note="Description of Artificial Sequence: Synthetic polypeptide"
QVQLKESGPGLVAPSQSLSITCTVSGFSLTNYGVSWVRQPPGKGLEWLGIIWGDGSTNYHSALISRLSISKDNSKSQVFLKLNSLQADDTATYYCAKPNWDTYAMDFWGQGTSVTVSS

SEQ ID NO: 126 - protein, 107 aa, Artificial Sequence
  source: /note="Description of Artificial Sequence: Synthetic polypeptide"
DIQMTQTTSSLSASLGDRVTISCRASQDISNFLNWYQQKPDGTVKLLIYCTSKLHSGVPSRFSGSGSETDYSLTISNLEQEDIATYFCQQGNTLPPTFGGGTKLEII

SEQ ID NO: 127 - protein, 120 aa, Artificial Sequence
  source: /note="Description of Artificial Sequence: Synthetic polypeptide"
EVQLQQSGPDLVKPGASVKISCKASGYSFTGYYMHWVKQSHGKSLEWIGRVYPNNGDTSYNQKFKVKAILTVDKSSSTAYMELRSLTSEDSAVYYCARGATVVESLFAYWGQGTLVTVSA

SEQ ID NO: 128 - protein, 111 aa, Artificial Sequence
  source: /note="Description of Artificial Sequence: Synthetic polypeptide"
DIVLTQSPASLAVSLGQRATISCRASESVDNYGNNFLHWYQQKPGQPPKLLIYRTSNLESGIPARFSGSGSRTDFTLTINPVEADDVATYYCQQSNEDPYTFGGGTKLEIK

SEQ ID NO: 129 - protein, 120 aa, Artificial Sequence
  source: /note="Description of Artificial Sequence: Synthetic polypeptide"
QIQLVQSGPELKKPGETVKISCKASGYTFTNYGMNWVKQAPGKGLKWMGWINTYIGEPIYADDFKGRFAFSLETSASTAYLQINNLKNEDMATYFCARRSDYDGYAMDYWGQGTSVTVSS

SEQ ID NO: 130 - protein, 112 aa, Artificial Sequence
  source: /note="Description of Artificial Sequence: Synthetic polypeptide"
DIVMSQSPSSLAVSVGERVTMSCKSSQSLLYSGNQKNYLAWYQQKPGQSPKLLIYWASTRESGVPDRFTGSGSGTDFTLTISSVKAEDLAVYYCQQHDSYPTFGGGSRLEIK

SEQ ID NO: 131 - protein, 122 aa, Artificial Sequence
  source: /note="Description of Artificial Sequence: Synthetic polypeptide"
EVQLQQSGPELVKPGASVKISCKASGYTFTDYYMNWVKQSHGKSLEWIGDFNPNNGGTTYNQKFEGKATLTVDKSSNTAYMDLRSLTSEDSAVYYCARGRFYYGSLYSFDYWGQGTTLTVSS

SEQ ID NO: 132 - protein, 106 aa, Artificial Sequence
  source: /note="Description of Artificial Sequence: Synthetic polypeptide"
DIQMTQSPASLSASVGETVTITCRASGNIHNYLAWYQQKQGKSPHLLVYNAKTLADGVPSRFSGSGSGTQYSLKINNLQPEDFGSYYCQHFWTSITFGAGTKLDLK

SEQ ID NO: 133 - protein, 122 aa, Artificial Sequence
  source: /note="Description of Artificial Sequence: Synthetic polypeptide"
QVQLVQSGAEVKKPGASVKVSCKASGYTFTDYYMNWVRQAPGQRLEWIGDFNPNNAGTTYNQKFEGRVTITVDKSASTAYMELSSLRSEDTAVYYCARGRFYYGSLYSFDYWGQGTLVTVSS

SEQ ID NO: 134 - protein, 106 aa, Artificial Sequence
  source: /note="Description of Artificial Sequence: Synthetic polypeptide"
DIQMTQSPSSLSASVGDRVTITCRASGNIHNYLAWYQQKPGKAPKLLIYNAKTLADGVPSRFSGSGSGTDFTLTISSLQPEDFATYYCQHFWTSITFGPGTKVDIK

SEQ ID NO: 135 - protein, 127 aa, Artificial Sequence
  source: /note="Description of Artificial Sequence: Synthetic polypeptide"
EVQLVESGGGLVQPKGSLKLSCAASGFTFNTYAMHWVRQAPGKGLEWVARIRSKSSNYATYYADSVKDRFTISRDDSQSMLYLQMNNLKTEDTAMYYCVRDGIYYYGTMYYYAMDYWGQGTSVTVSS

SEQ ID NO: 136 - protein, 111 aa, Artificial Sequence
  source: /note="Description of Artificial Sequence: Synthetic polypeptide"
NIVLTQSPASLAVSLGQRATISCRASESVDYYGNSFMYWYQQKPGQPPKLLIYFASNLESGVPARFSGSGSRTDFTLTIDPVEAADAASYYCQQNNEDPWTFGGGTKLEIK

SEQ ID NO: 137 - protein, 127 aa, Artificial Sequence
  source: /note="Description of Artificial Sequence: Synthetic polypeptide"
EVQLVESGGGLVQPKGSLKLSCAASGFTFNTYAMHWVRQAPGKGLEWVARIRSKSSNYATYYADSVKDRFTISRDDSQSMLYLQMNNLKTEDTAMYYCVRDGIYYYDTMYYYAMDYWGQGTSVTVSS

SEQ ID NO: 138 - protein, 111 aa, Artificial Sequence
  source: /note="Description of Artificial Sequence: Synthetic polypeptide"
NIVLTQSPASLAVSLGQRATISCRASESVDYYGNSFIYWYQQKPGQPPKLLIYFASNLESGVPARFSGSGSRTDFTLTIDPVEAADAASYYCQQNNEDPWTFGGGTKLEIK

SEQ ID NO: 139 - protein, 127 aa, Artificial Sequence
  source: /note="Description of Artificial Sequence: Synthetic polypeptide"
EVQLVESGGGLVQPGGSLRLSCAASGFTFNTYAMHWVRQAPGKGLEWVARIRSKSSNYATYYADSVKDRFTISRDDAKNSLYLQMNSLRAEDTAVYYCARDGIYYYDTMYYYAMDYWGQGTLVTVSS

SEQ ID NO: 140 - protein, 111 aa, Artificial Sequence
  source: /note="Description of Artificial Sequence: Synthetic polypeptide"
NIVLTQSPDSLAVSLGERATINCRASESVDYYGNSFIYWYQQKPGQPPKLLIYFASNLESGVPDRFSGSGSGTDFTLTISSLQAEDVAVYYCQQNNEDPWTFGGGTKVEIK

SEQ ID NO: 141 - protein, 125 aa, Artificial Sequence
  source: /note="Description of Artificial Sequence: Synthetic polypeptide"
AVQLQQSGPELVKPGASVKISCKASGYTFTDYYMNWVKQSHGKSLEWIGNVNPNNGGTSYNQKFKGKATLTVDKSSSTAYMELRSLTSEDSAVYYCARREIYFYGTIYYYAMDYWGQGTSVTVSS

SEQ ID NO: 142 - protein, 111 aa, Artificial Sequence
  source: /note="Description of Artificial Sequence: Synthetic polypeptide"
DIVLTQSPASLAVSLGQRATISCRASESVDYYGNSFMYWYQQKPGRPPNLLIYFASNLESGVPARFSGSGSRTDFTLTIDPVEADDAATYYCQQNNEDPWTFGGGTKLEIK

SEQ ID NO: 143 - protein, 125 aa, Artificial Sequence
  source: /note="Description of Artificial Sequence: Synthetic polypeptide"
AVQLQQSGPELVKPGASVKISCKASGYTFTDYYINWVKQSHGKSLQWIGNVNPNDGGTTYNQKFKGKATLTVDKSSSTAYMELRSLTSEDSAVYYCARREIYFYGTIYYYAMDYWGQGTSVTVSS

SEQ ID NO: 144 - protein, 125 aa, Artificial Sequence
  source: /note="Description of Artificial Sequence: Synthetic polypeptide"
QVQLVQSGAEVKKPGASVKVSCKASGYTFTDYYINWVRQAPGQGLEWMGNVNPNDGGTTYNQKFKGRVTMTTDTSTSTAYMELRSLRSDDTAVYYCARREIYFYGTIYYYAMDYWGQGTLVTVSS

SEQ ID NO: 145 - protein, 111 aa, Artificial Sequence
  source: /note="Description of Artificial Sequence: Synthetic polypeptide"
DIQLTQSPSFLSASVGDRVTITCRASESVDYYGNSFMYWYQQKPGKAPKLLIYFASNLESGVPSRFSGSGSGTEFTLTISSLQPEDFATYYCQQNNEDPWTFGGGTKVEIK

SEQ ID NO: 146 - protein, 474 aa, Artificial Sequence
  source: /note="Description of Artificial Sequence: Synthetic polypeptide"
MDMRVPAQLLGLLLLWLRGARCQVQLVQSGAEVKKPGASVKVSCKASGYTFTDYYMNWVRQAPGQRLEWIGDFNPNNAGTTYNQKFEGRVTITVDKSASTAYMELSSLRSEDTAVYYCARGRFYYGSLYSFDYWGQGTLVTVSSASTKGPSVFPLAPSSKSTSGGTAALGCLVKDYFPEPVTVSWNSGALTSGVHTFPAVLQSSGLYSLSSVVTVPSSSLGTQTYICNVNHKPSNTKVDKKVEPKSCDKTHTCPPCPAPELLGGPSVFLFPPKPKDTLMISRTPEVTCVVVDVSHEDPEVKFNWYVDGVEVHNAKTKPREEQYGSTYRVVSVLTVLHQDWLNGKEYKCKVSNKALPAPIEKTISKAKGQPREPQVYTLPPSREEMTKNQVSLTCLVKGFYPSDIAVEWESNGQPENNYKTTPPVLDSDGSFFLYSKLTVDKSRWQQGNVFSCSVMHEALHNHYTQKSLSLSPGK

SEQ ID NO: 147 - protein, 235 aa, Artificial Sequence
  source: /note="Description of Artificial Sequence: Synthetic polypeptide"
MDMRVPAQLLGLLLLWLRGARCDIQMTQSPSSLSASVGDRVTITCRASGNIHNYLAWYQQKPGKAPKLLIYNAKTLADGVPSRFSGSGSGTDFTLTISSLQPEDFATYYCQHFWTSITFGPGTKVDIKRTVAAPSVFIFPPSDEQLKSGTASVVCLLNNFYPREAKVQWKVDNALQSGNSQESVTEQDSKDSTYSLSSTLTLSKADYEKHKVYACEVTHQGLSSPVTKSFNRGEC

SEQ ID NO: 148 - protein, 452 aa, Artificial Sequence
  source: /note="Description of Artificial Sequence: Synthetic polypeptide"
QVQLVQSGAEVKKPGASVKVSCKASGYTFTDYYMNWVRQAPGQRLEWIGDFNPNNAGTTYNQKFEGRVTITVDKSASTAYMELSSLRSEDTAVYYCARGRFYYGSLYSFDYWGQGTLVTVSSASTKGPSVFPLAPSSKSTSGGTAALGCLVKDYFPEPVTVSWNSGALTSGVHTFPAVLQSSGLYSLSSVVTVPSSSLGTQTYICNVNHKPSNTKVDKKVEPKSCDKTHTCPPCPAPELLGGPSVFLFPPKPKDTLMISRTPEVTCVVVDVSHEDPEVKFNWYVDGVEVHNAKTKPREEQYGSTYRVVSVLTVLHQDWLNGKEYKCKVSNKALPAPIEKTISKAKGQPREPQVYTLPPSREEMTKNQVSLTCLVKGFYPSDIAVEWESNGQPENNYKTTPPVLDSDGSFFLYSKLTVDKSRWQQGNVFSCSVMHEALHNHYTQKSLSLSPGK

SEQ ID NO: 149 - protein, 213 aa, Artificial Sequence
  source: /note="Description of Artificial Sequence: Synthetic polypeptide"
DIQMTQSPSSLSASVGDRVTITCRASGNIHNYLAWYQQKPGKAPKLLIYNAKTLADGVPSRFSGSGSGTDFTLTISSLQPEDFATYYCQHFWTSITFGPGTKVDIKRTVAAPSVFIFPPSDEQLKSGTASVVCLLNNFYPREAKVQWKVDNALQSGNSQESVTEQDSKDSTYSLSSTLTLSKADYEKHKVYACEVTHQGLSSPVTKSFNRGEC

SEQ ID NO: 150 - protein, 479 aa, Artificial Sequence
  source: /note="Description of Artificial Sequence: Synthetic polypeptide"
MDMRVPAQLLGLLLLWLRGARCEVQLVESGGGLVQPGGSLRLSCAASGFTFNTYAMHWVRQAPGKGLEWVARIRSKSSNYATYYADSVKDRFTISRDDAKNSLYLQMNSLRAEDTAVYYCARDGIYYYDTMYYYAMDYWGQGTLVTVSSASTKGPSVFPLAPSSKSTSGGTAALGCLVKDYFPEPVTVSWNSGALTSGVHTFPAVLQSSGLYSLSSVVTVPSSSLGTQTYICNVNHKPSNTKVDKKVEPKSCDKTHTCPPCPAPELLGGPSVFLFPPKPKDTLMISRTPEVTCVVVDVSHEDPEVKFNWYVDGVEVHNAKTKPREEQYGSTYRVVSVLTVLHQDWLNGKEYKCKVSNKALPAPIEKTISKAKGQPREPQVYTLPPSREEMTKNQVSLTCLVKGFYPSDIAVEWESNGQPENNYKTTPPVLDSDGSFFLYSKLTVDKSRWQQGNVFSCSVMHEALHNHYTQKSLSLSPGK

SEQ ID NO: 151 - protein, 240 aa, Artificial Sequence
  source: /note="Description of Artificial Sequence: Synthetic polypeptide"
MDMRVPAQLLGLLLLWLRGARCNIVLTQSPDSLAVSLGERATINCRASESVDYYGNSFIYWYQQKPGQPPKLLIYFASNLESGVPDRFSGSGSGTDFTLTISSLQAEDVAVYYCQQNNEDPWTFGGGTKVEIKRTVAAPSVFIFPPSDEQLKSGTASVVCLLNNFYPREAKVQWKVDNALQSGNSQESVTEQDSKDSTYSLSSTLTLSKADYEKHKVYACEVTHQGLSSPVTKSFNRGEC

SEQ ID NO: 152 - protein, 457 aa, Artificial Sequence
  source: /note="Description of Artificial Sequence: Synthetic polypeptide"
EVQLVESGGGLVQPGGSLRLSCAASGFTFNTYAMHWVRQAPGKGLEWVARIRSKSSNYATYYADSVKDRFTISRDDAKNSLYLQMNSLRAEDTAVYYCARDGIYYYDTMYYYAMDYWGQGTLVTVSSASTKGPSVFPLAPSSKSTSGGTAALGCLVKDYFPEPVTVSWNSGALTSGVHTFPAVLQSSGLYSLSSVVTVPSSSLGTQTYICNVNHKPSNTKVDKKVEPKSCDKTHTCPPCPAPELLGGPSVFLFPPKPKDTLMISRTPEVTCVVVDVSHEDPEVKFNWYVDGVEVHNAKTKPREEQYGSTYRVVSVLTVLHQDWLNGKEYKCKVSNKALPAPIEKTISKAKGQPREPQVYTLPPSREEMTKNQVSLTCLVKGFYPSDIAVEWESNGQPENNYKTTPPVLDSDGSFFLYSKLTVDKSRWQQGNVFSCSVMHEALHNHYTQKSLSLSPGK

SEQ ID NO: 153 - protein, 218 aa, Artificial Sequence
  source: /note="Description of Artificial Sequence: Synthetic polypeptide"
NIVLTQSPDSLAVSLGERATINCRASESVDYYGNSFIYWYQQKPGQPPKLLIYFASNLESGVPDRFSGSGSGTDFTLTISSLQAEDVAVYYCQQNNEDPWTFGGGTKVEIKRTVAAPSVFIFPPSDEQLKSGTASVVCLLNNFYPREAKVQWKVDNALQSGNSQESVTEQDSKDSTYSLSSTLTLSKADYEKHKVYACEVTHQGLSSPVTKSFNRGEC

SEQ ID NO: 154 - protein, 477 aa, Artificial Sequence
  source: /note="Description of Artificial Sequence: Synthetic polypeptide"
MDMRVPAQLLGLLLLWLRGARCQVQLVQSGAEVKKPGASVKVSCKASGYTFTDYYINWVRQAPGQGLEWMGNVNPNDGGTTYNQKFKGRVTMTTDTSTSTAYMELRSLRSDDTAVYYCARREIYFYGTIYYYAMDYWGQGTLVTVSSASTKGPSVFPLAPSSKSTSGGTAALGCLVKDYFPEPVTVSWNSGALTSGVHTFPAVLQSSGLYSLSSVVTVPSSSLGTQTYICNVNHKPSNTKVDKKVEPKSCDKTHTCPPCPAPELLGGPSVFLFPPKPKDTLMISRTPEVTCVVVDVSHEDPEVKFNWYVDGVEVHNAKTKPREEQYGSTYRVVSVLTVLHQDWLNGKEYKCKVSNKALPAPIEKTISKAKGQPREPQVYTLPPSREEMTKNQVSLTCLVKGFYPSDIAVEWESNGQPENNYKTTPPVLDSDGSFFLYSKLTVDKSRWQQGNVFSCSVMHEALHNHYTQKSLSLSPGK

SEQ ID NO: 155 - protein, 240 aa, Artificial Sequence
  source: /note="Description of Artificial Sequence: Synthetic polypeptide"
MDMRVPAQLLGLLLLWLRGARCDIQLTQSPSFLSASVGDRVTITCRASESVDYYGNSFMYWYQQKPGKAPKLLIYFASNLESGVPSRFSGSGSGTEFTLTISSLQPEDFATYYCQQNNEDPWTFGGGTKVEIKRTVAAPSVFIFPPSDEQLKSGTASVVCLLNNFYPREAKVQWKVDNALQSGNSQESVTEQDSKDSTYSLSSTLTLSKADYEKHKVYACEVTHQGLSSPVTKSFNRGEC

SEQ ID NO: 156 - protein, 455 aa, Artificial Sequence
  source: /note="Description of Artificial Sequence: Synthetic polypeptide"
QVQLVQSGAEVKKPGASVKVSCKASGYTFTDYYINWVRQAPGQGLEWMGNVNPNDGGTTYNQKFKGRVTMTTDTSTSTAYMELRSLRSDDTAVYYCARREIYFYGTIYYYAMDYWGQGTLVTVSSASTKGPSVFPLAPSSKSTSGGTAALGCLVKDYFPEPVTVSWNSGALTSGVHTFPAVLQSSGLYSLSSVVTVPSSSLGTQTYICNVNHKPSNTKVDKKVEPKSCDKTHTCPPCPAPELLGGPSVFLFPPKPKDTLMISRTPEVTCVVVDVSHEDPEVKFNWYVDGVEVHNAKTKPREEQYGSTYRVVSVLTVLHQDWLNGKEYKCKVSNKALPAPIEKTISKAKGQPREPQVYTLPPSREEMTKNQVSLTCLVKGFYPSDIAVEWESNGQPENNYKTTPPVLDSDGSFFLYSKLTVDKSRWQQGNVFSCSVMHEALHNHYTQKSLSLSPGK

SEQ ID NO: 157 - protein, 218 aa, Artificial Sequence
  source: /note="Description of Artificial Sequence: Synthetic polypeptide"
DIQLTQSPSFLSASVGDRVTITCRASESVDYYGNSFMYWYQQKPGKAPKLLIYFASNLESGVPSRFSGSGSGTEFTLTISSLQPEDFATYYCQQNNEDPWTFGGGTKVEIKRTVAAPSVFIFPPSDEQLKSGTASVVCLLNNFYPREAKVQWKVDNALQSGNSQESVTEQDSKDSTYSLSSTLTLSKADYEKHKVYACEVTHQGLSSPVTKSFNRGEC

SEQ ID NO: 158 - protein, 330 aa, Homo sapiens
ASTKGPSVFPLAPSSKSTSGGTAALGCLVKDYFPEPVTVSWNSGALTSGVHTFPAVLQSSGLYSLSSVVTVPSSSLGTQTYICNVNHKPSNTKVDKKVEPKSCDKTHTCPPCPAPELLGGPSVFLFPPKPKDTLMISRTPEVTCVVVDVSHEDPEVKFNWYVDGVEVHNAKTKPREEQYNSTYRVVSVLTVLHQDWLNGKEYKCKVSNKALPAPIEKTISKAKGQPREPQVYTLPPSREEMTKNQVSLTCLVKGFYPSDIAVEWESNGQPENNYKTTPPVLDSDGSFFLYSKLTVDKSRWQQGNVFSCSVMHEALHNHYTQKSLSLSPGK

SEQ ID NO: 159 - protein, 330 aa, Artificial Sequence
  source: /note="Description of Artificial Sequence: Synthetic polypeptide"
ASTKGPSVFPLAPSSKSTSGGTAALGCLVKDYFPEPVTVSWNSGALTSGVHTFPAVLQSSGLYSLSSVVTVPSSSLGTQTYICNVNHKPSNTKVDKKVEPKSCDKTHTCPPCPAPALAGGPSVFLFPPKPKDTLMISRTPEVTCVVVDVSHEDPEVKFNWYVDGVEVHNAKTKPREEQYNSTYRVVSVLTVLHQDWLNGKEYKCKVSNKALPAPIEKTISKAKGQPREPQVYTLPPSREEMTKNQVSLTCLVKGFYPSDIAVEWESNGQPENNYKTTPPVLDSDGSFFLYSKLTVDKSRWQQGNVFSCSVMHEALHNHYTQKSLSLSPGK

SEQ ID NO: 160 - protein, 330 aa, Artificial Sequence
  source: /note="Description of Artificial Sequence: Synthetic polypeptide"
ASTKGPSVFPLAPSSKSTSGGTAALGCLVKDYFPEPVTVSWNSGALTSGVHTFPAVLQSSGLYSLSSVVTVPSSSLGTQTYICNVNHKPSNTKVDKKVEPKSCDKTHTCPPCPAPEAAGGPSVFLFPPKPKDTLMISRTPEVTCVVVDVSHEDPEVKFNWYVDGVEVHNAKTKPREEQYNSTYRVVSVLTVLHQDWLNGKEYKCKVSNKALPAPIEKTISKAKGQPREPQVYTLPPSREEMTKNQVSLTCLVKGFYPSDIAVEWESNGQPENNYKTTPPVLDSDGSFFLYSKLTVDKSRWQQGNVFSCSVMHEALHNHYTQKSLSLSPGK

SEQ ID NO: 161 - protein, 330 aa, Artificial Sequence
  source: /note="Description of Artificial Sequence: Synthetic polypeptide"
ASTKGPSVFPLAPSSKSTSGGTAALGCLVKDYFPEPVTVSWNSGALTSGVHTFPAVLQSSGLYSLSSVVTVPSSSLGTQTYICNVNHKPSNTKVDKKVEPKSCDKTHTCPPCPAPEAAGGPSVFLFPPKPKDTLMISRTPEVTCVVVDVSHEDPEVKFNWYVDGVEVHNAKTKPREEQYNSTYRVVSVLTVLHQDWLNGKEYKCKVSNKALGAPIEKTISKAKGQPREPQVYTLPPSREEMTKNQVSLTCLVKGFYPSDIAVEWESNGQPENNYKTTPPVLDSDGSFFLYSKLTVDKSRWQQGNVFSCSVMHEALHNHYTQKSLSLSPGK

SEQ ID NO: 162 - protein, 330 aa, Artificial Sequence
  source: /note="Description of Artificial Sequence: Synthetic polypeptide"
ASTKGPSVFPLAPSSKSTSGGTAALGCLVKDYFPEPVTVSWNSGALTSGVHTFPAVLQSSGLYSLSSVVTVPSSSLGTQTYICNVNHKPSNTKVDKKVEPKSCDKTHTCPPCPAPELLGGPSVFLFPPKPKDTLMISRTPEVTCVVVDVSHEDPEVKFNWYVDGVEVHNAKTKPREEQYGSTYRVVSVLTVLHQDWLNGKEYKCKVSNKALPAPIEKTISKAKGQPREPQVYTLPPSREEMTKNQVSLTCLVKGFYPSDIAVEWESNGQPENNYKTTPPVLDSDGSFFLYSKLTVDKSRWQQGNVFSCSVMHEALHNHYTQKSLSLSPGK

SEQ ID NO: 163 - protein, 330 aa, Artificial Sequence
  source: /note="Description of Artificial Sequence: Synthetic polypeptide"
ASTKGPSVFPLAPSSKSTSGGTAALGCLVKDYFPEPVTVSWNSGALTSGVHTFPAVLQSSGLYSLSSVVTVPSSSLGTQTYICNVNHKPSNTKVDKKVEPKSCDKTHTCPPCPAPELLGGPSVFLFPPKPKDTLMISRTPEVTCVVVDVSHEDPEVKFNWYVDGVEVHNAKTKPREEQYGSTYRVVSVLTVLAQDWLNGKEYKCKVSNKALPAPIEKTISKAKGQPREPQVYTLPPSREEMTKNQVSLTCLVKGFYPSDIAVEWESNGQPENNYKTTPPVLDSDGSFFLYSKLTVDKSRWQQGNVFSCSVMHEALHNHYTQKSLSLSPGK

SEQ ID NO: 164 - protein, 107 aa, Artificial Sequence [sequence omitted]

SEQ ID NO: 165 - protein, 106 aa, Artificial Sequence
  source: /note="Description of Artificial Sequence: Synthetic polypeptide"
GQPKAAPSVTLFPPSSEELQANKATLVCLISDFYPGAVTVAWKADSSPVKAGVETTTPSKQSNNKYAASSYLSLTPEQWKSHRSYSCQVTHEGSTVEKTVAPTECS

SEQ ID NO: 166 - protein, 651 aa, Macaca fascicularis
MTPILMVLICLGLSLGPRTHVQAGILPKPTLWAEPGSMISEGSPVTLRCQGSLQVQEYRLYREKKPASWVRRIQQELVKKGYFAIGFITWEHTGQYRCQYYSHSWWSEPSDPLELVVTGAYSKPTLSALPSPVVASGGNVTLQCDSQVAFDSFTLCKEGEDEHPQRLNCQSHARGWSWAVFSVGPVSPSRRWSYRCYGYISSAPNVWSLPSDLLELLVPGVSKKPSLSVQPGPVVAPGDKLTLQCGSDAGYDRFALYKEGEGDFLQRPVRQPQAGLSQANFLLGPVSRSHGGQYRCSGAHNLSSEWSAPSDPLDILIAGQIRGRPFLSVQPGPKVVSGENVTLLCQSSWQFHAFLLTQAGAADAHLHLRSMYKYPKYQAEFPMSPVTSAHAGTYRCYGSRSSNPYLLSVPSDPLELVVSGPSGGPSSPTTGPTSTCAGPEDQPLTPTGSDPQSGLGRHLGVVTGILVAFVLLLFLLLLLFLVLRHQRQGKHWTSAQRKADFQHPAGAVEPEPRDRGLQRRSSPAADTQEENLYAAVKDTQPEDGVELDSRQRPHDEDPQAVTYARVKHSRPRREMASPPSPLSEEFLDTKDTQAEEDRQMDTEAAASEDPQDVTYAQLQSLTLRRETTEPPPSQERAPPVESSIYATLTIH

SEQ ID NO: 167 - protein, 628 aa, Macaca fascicularis
GILPKPTLWAEPGSMISEGSPVTLRCQGSLQVQEYRLYREKKPASWVRRIQQELVKKGYFAIGFITWEHTGQYRCQYYSHSWWSEPSDPLELVVTGAYSKPTLSALPSPVVASGGNVTLQCDSQVAFDSFTLCKEGEDEHPQRLNCQSHARGWSWAVFSVGPVSPSRRWSYRCYGYISSAPNVWSLPSDLLELLVPGVSKKPSLSVQPGPVVAPGDKLTLQCGSDAGYDRFALYKEGEGDFLQRPVRQPQAGLSQANFLLGPVSRSHGGQYRCSGAHNLSSEWSAPSDPLDILIAGQIRGRPFLSVQPGPKVVSGENVTLLCQSSWQFHAFLLTQAGAADAHLHLRSMYKYPKYQAEFPMSPVTSAHAGTYRCYGSRSSNPYLLSVPSDPLELVVSGPSGGPSSPTTGPTSTCAGPEDQPLTPTGSDPQSGLGRHLGVVTGILVAFVLLLFLLLLLFLVLRHQRQGKHWTSAQRKADFQHPAGAVEPEPRDRGLQRRSSPAADTQEENLYAAVKDTQPEDGVELDSRQRPHDEDPQAVTYARVKHSRPRREMASPPSPLSEEFLDTKDTQAEEDRQMDTEAAASEDPQDVTYAQLQSLTLRRETTEPPPSQERAPPVESSIYATLTIH

SEQ ID NO: 168 - protein, 438 aa, Macaca fascicularis
GILPKPTLWAEPGSMISEGSPVTLRCQGSLQVQEYRLYREKKPASWVRRIQQELVKKGYFAIGFITWEHTGQYRCQYYSHSWWSEPSDPLELVVTGAYSKPTLSALPSPVVASGGNVTLQCDSQVAFDSFTLCKEGEDEHPQRLNCQSHARGWSWAVFSVGPVSPSRRWSYRCYGYISSAPNVWSLPSDLLELLVPGVSKKPSLSVQPGPVVAPGDKLTLQCGSDAGYDRFALYKEGEGDFLQRPVRQPQAGLSQANFLLGPVSRSHGGQYRCSGAHNLSSEWSAPSDPLDILIAGQIRGRPFLSVQPGPKVVSGENVTLLCQSSWQFHAFLLTQAGAADAHLHLRSMYKYPKYQAEFPMSPVTSAHAGTYRCYGSRSSNPYLLSVPSDPLELVVSGPSGGPSSPTTGPTSTCAGPEDQPLTPTGSDPQSGLGRHLGV

SEQ ID NO: 169 - protein, 88 aa, Macaca fascicularis
PKPTLWAEPGSMISEGSPVTLRCQGSLQVQEYRLYREKKPASWVRRIQQELVKKGYFAIGFITWEHTGQYRCQYYSHSWWSEPSDPLE

SEQ ID NO: 170 - protein, 106 aa, Macaca fascicularis
LVVTGAYSKPTLSALPSPVVASGGNVTLQCDSQVAFDSFTLCKEGEDEHPQRLNCQSHARGWSWAVFSVGPVSPSRRWSYRCYGYISSAPNVWSLPSDLLELLVPG

SEQ ID NO: 171 - protein, 91 aa, Macaca fascicularis
VSKKPSLSVQPGPVVAPGDKLTLQCGSDAGYDRFALYKEGEGDFLQRPVRQPQAGLSQANFLLGPVSRSHGGQYRCSGAHNLSSEWSAPSD

SEQ ID NO: 172 - protein, 97 aa, Macaca fascicularis
PLDILIAGQIRGRPFLSVQPGPKVVSGENVTLLCQSSWQFHAFLLTQAGAADAHLHLRSMYKYPKYQAEFPMSPVTSAHAGTYRCYGSRSSNPYLLS

SEQ ID NO: 173 - protein, 6 aa, Artificial Sequence
  source: /note="Description of Artificial Sequence: Synthetic 6xHis tag"
HHHHHH